European Patent Specification EP 3 472 190 B1, published October 11, 2023. Title: FIBRONECTIN-BINDING PEPTIDES FOR USE IN TUMOR OR FIBROSIS DIAGNOSIS AND THERAPY. Applicant: ETH Zurich, PSI Villigen. The sequence listing filed with the application follows.

SEQUENCE LISTING (296 sequences)

SEQ ID NO: 1 - protein, 7 aa, Streptococcus pyogenes
TEVYGNQ

SEQ ID NO: 2 - protein, 7 aa, Streptococcus pyogenes
VDIDKKL

SEQ ID NO: 3 - protein, 7 aa, Streptococcus pyogenes
PNETGFS

SEQ ID NO: 4 - protein, 7 aa, Streptococcus pyogenes
MVETEDT

SEQ ID NO: 5 - protein, 7 aa, Streptococcus pyogenes
EVLMGGQ

SEQ ID NO: 6 - protein, 7 aa, Streptococcus pyogenes
VEFTKDT

SEQ ID NO: 7 - protein, 7 aa, Streptococcus pyogenes
TGMSGQT

SEQ ID NO: 8 - protein, 7 aa, Streptococcus pyogenes
QVETEDT

SEQ ID NO: 9 - protein, 7 aa, Streptococcus pyogenes
GVLMGGQ

SEQ ID NO: 10 - protein, 7 aa, Streptococcus pyogenes
TGMSGFS

SEQ ID NO: 11 - protein, 7 aa, Streptococcus pyogenes
VTIIEDT

SEQ ID NO: 12 - protein, 7 aa, Streptococcus pyogenes
LVFHFDN

SEQ ID NO: 13 - protein, 7 aa, Streptococcus pyogenes
VSTQENK

SEQ ID NO: 14 - protein, 7 aa, Streptococcus pyogenes
VDITEDT

SEQ ID NO: 15 - protein, 7 aa, Streptococcus pyogenes
PGMSGSN

SEQ ID NO: 16 - protein, 7 aa, Streptococcus pyogenes
TVVEEDT

SEQ ID NO: 17 - protein, 7 aa, Streptococcus pyogenes
DVLVGGQ

SEQ ID NO: 18 - protein, 7 aa, Streptococcus pyogenes
IDITEDT

SEQ ID NO: 19 - protein, 7 aa, Streptococcus pyogenes
DILVGGQ

SEQ ID NO: 20 - protein, 7 aa, Streptococcus pyogenes
TVIEEDT

SEQ ID NO: 21 - protein, 7 aa, Streptococcus pyogenes
RFFHFDN

SEQ ID NO: 22 - protein, 7 aa, Streptococcus pyogenes
REVITQQ

SEQ ID NO: 23 - protein, 7 aa, Streptococcus pyogenes
NLEIEET

SEQ ID NO: 24 - protein, 7 aa, Streptococcus pyogenes
PLESGAS

SEQ ID NO: 25 - protein, 7 aa, Streptococcus pyogenes
TTTVEDS

SEQ ID NO: 26 - protein, 7 aa, Streptococcus pyogenes
YKPTKGS

SEQ ID NO: 27 - protein, 7 aa, Streptococcus pyogenes
VIDIEEK

SEQ ID NO: 28 - protein, 7 aa, Streptococcus pyogenes
PDEQGHS

SEQ ID NO: 29 - protein, 7 aa, Streptococcus pyogenes
TTEIEDS

SEQ ID NO: 30 - protein, 7 aa, Streptococcus pyogenes
DVIIGGQ

SEQ ID NO: 31 - protein, 7 aa, Streptococcus pyogenes
VDTTEDT

SEQ ID NO: 32 - protein, 7 aa, Streptococcus pyogenes
SGMTGHS

SEQ ID NO: 33 - protein, 7 aa, Streptococcus pyogenes
VETTEDT

SEQ ID NO: 34 - protein, 7 aa, Streptococcus pyogenes
TGMHGDS

SEQ ID NO: 35 - protein, 7 aa, Streptococcus pyogenes
KTEVEDT

SEQ ID NO: 36 - protein, 7 aa, Streptococcus pyogenes
QLFHFDN

SEQ ID NO: 37 - protein, 7 aa, Streptococcus equi
PGQTGGQ

SEQ ID NO: 38 - protein, 7 aa, Streptococcus equi
IETTEDT

SEQ ID NO: 39 - protein, 7 aa, Streptococcus equi
KGMSGQS

SEQ ID NO: 40 - protein, 7 aa, Streptococcus equi
TIESENT

SEQ ID NO: 41 - protein, 7 aa, Streptococcus equi
EVMIGGQ

SEQ ID NO: 42 - protein, 7 aa, Streptococcus equi
TIESEDT

SEQ ID NO: 43 - protein, 7 aa, Streptococcus equi
IDFSENT

SEQ ID NO: 44 - protein, 7 aa, Streptococcus equi
SGMSGQS

SEQ ID NO: 45 - protein, 7 aa, Streptococcus equi
TTVIEDT

SEQ ID NO: 46 - protein, 7 aa, Streptococcus equi
EIIIGGQ

SEQ ID NO: 47 - protein, 7 aa, Streptococcus equi
IDFSEDT

SEQ ID NO: 48 - protein, 7 aa, Streptococcus equi
PGMSGQS

SEQ ID NO: 49 - protein, 7 aa, Streptococcus equi
TTIVEDT

SEQ ID NO: 50 - protein, 7 aa, Streptococcus dysgalactiae
ENNLGGQ

SEQ ID NO: 51 - protein, 7 aa, Streptococcus dysgalactiae
ITITEDS

SEQ ID NO: 52 - protein, 7 aa, Streptococcus dysgalactiae
SGMSGQN

SEQ ID NO: 53 - protein, 7 aa, Streptococcus dysgalactiae
ETVVEDT

SEQ ID NO: 54 - protein, 7 aa, Streptococcus dysgalactiae
DIVLGGP

SEQ ID NO: 55 - protein, 7 aa, Streptococcus dysgalactiae
IDFTEDS

SEQ ID NO: 56 - protein, 7 aa, Streptococcus dysgalactiae
PGMSGNN

SEQ ID NO: 57 - protein, 7 aa, Streptococcus dysgalactiae
HTITEDS

SEQ ID NO: 58 - protein, 7 aa, Streptococcus dysgalactiae
EVIIGGQ

SEQ ID NO: 59 - protein, 7 aa, Streptococcus dysgalactiae
IDFTEDT

SEQ ID NO: 60 - protein, 7 aa, Streptococcus dysgalactiae
SGMSGDN

SEQ ID NO: 61 - protein, 7 aa, Streptococcus dysgalactiae
TVLEEDS

SEQ ID NO: 62 - protein, 7 aa, Streptococcus dysgalactiae
TGMSGAG

SEQ ID NO: 63 - protein, 7 aa, Streptococcus dysgalactiae
PTITEET

SEQ ID NO: 64 - protein, 7 aa, Streptococcus dysgalactiae
EIIMGGQ

SEQ ID NO: 65 - protein, 7 aa, Streptococcus dysgalactiae
IDMVEDT

SEQ ID NO: 66 - protein, 7 aa, Streptococcus dysgalactiae
PGMSGSN

SEQ ID NO: 67 - protein, 7 aa, Streptococcus dysgalactiae
TVVEEDT

SEQ ID NO: 68 - protein, 7 aa, Streptococcus dysgalactiae
LQFHFDN

SEQ ID NO: 69 - protein, 7 aa, Streptococcus dysgalactiae
EVIIQQG

SEQ ID NO: 70 - protein, 7 aa, Streptococcus dysgalactiae
ILGLEET

SEQ ID NO: 71 - protein, 7 aa, Streptococcus dysgalactiae
PTEEHQS

SEQ ID NO: 72 - protein, 7 aa, Streptococcus dysgalactiae
TTTIEDT

SEQ ID NO: 73 - protein, 7 aa, Streptococcus dysgalactiae
DKPITEA

SEQ ID NO: 74 - protein, 7 aa, Streptococcus dysgalactiae
SIDFEET

SEQ ID NO: 75 - protein, 7 aa, Streptococcus dysgalactiae
PTEQGQS

SEQ ID NO: 76 - protein, 7 aa, Streptococcus dysgalactiae
TTEVEDT

SEQ ID NO: 77 - protein, 7 aa, Streptococcus dysgalactiae
IVDIEEN

SEQ ID NO: 78 - protein, 7 aa, Streptococcus dysgalactiae
VVDIEES

SEQ ID NO: 79 - protein, 7 aa, Streptococcus dysgalactiae
TTEVEDS

SEQ ID NO: 80 - protein, 7 aa, Streptococcus dysgalactiae
LSIHFDN

SEQ ID NO: 81 - protein, 7 aa, Staphylococcus aureus
GPIIQNN

SEQ ID NO: 82 - protein, 7 aa, Staphylococcus aureus
FEYKEDT

SEQ ID NO: 83 - protein, 7 aa, Staphylococcus aureus
ETLTGQY

SEQ ID NO: 84 - protein, 7 aa, Staphylococcus aureus
TTVEEEY

SEQ ID NO: 85 - protein, 6 aa, Staphylococcus aureus
IDFEES

SEQ ID NO: 86 - protein, 7 aa, Staphylococcus aureus
ENSKHHA

SEQ ID NO: 87 - protein, 7 aa, Staphylococcus aureus
VEYEEDT

SEQ ID NO: 88 - protein, 7 aa, Staphylococcus aureus
QVTTESN

SEQ ID NO: 89 - protein, 7 aa, Staphylococcus aureus
VEFDEES

SEQ ID NO: 90 - protein, 7 aa, Staphylococcus aureus
GIVTGAV

SEQ ID NO: 91 - protein, 7 aa, Staphylococcus aureus
HTTVEDT

SEQ ID NO: 92 - protein, 7 aa, Staphylococcus aureus
KYEQGGN

SEQ ID NO: 93 - protein, 7 aa, Staphylococcus aureus
VDIDFDS

SEQ ID NO: 94 - protein, 7 aa, Staphylococcus aureus
PQIHGQN

SEQ ID NO: 95 - protein, 7 aa, Staphylococcus aureus
QSFEEDT

SEQ ID NO: 96 - protein, 7 aa, Staphylococcus aureus
KYEHGGN

SEQ ID NO: 97 - protein, 7 aa, Staphylococcus aureus
IDIDFDS

SEQ ID NO: 98 - protein, 7 aa, Staphylococcus aureus
PHIHGFN

SEQ ID NO: 99 - protein, 7 aa, Staphylococcus aureus
EIIEEDT

SEQ ID NO: 100 - protein, 7 aa, Staphylococcus aureus
SYQFGGH

SEQ ID NO: 101 - protein, 7 aa, Staphylococcus aureus
VDFEEDT

SEQ ID NO: 102 - protein, 7 aa, Staphylococcus aureus
PKVSGQN

SEQ ID NO: 103 - protein, 7 aa, Staphylococcus aureus
QTIEEDT

SEQ ID NO: 104 - protein, 6 aa, Borrelia burgdorferi
EPIESN

SEQ ID NO: 105 - protein, 7 aa, Borrelia burgdorferi
IDLTIDS

SEQ ID NO: 106 - protein, 7 aa, Borrelia burgdorferi
QGIAGSN

SEQ ID NO: 107 - protein, 7 aa, Borrelia burgdorferi
EIEEEDY

SEQ ID NO: 108 - protein, 11 aa, Mycobacterium tuberculosis
FEWYDQSGLSV

SEQ ID NO: 109 - protein, 11 aa, Mycobacterium tuberculosis
FEWYYQSGLSI

SEQ ID NO: 110 - protein, 11 aa, Mycobacterium tuberculosis
FEEYYQSGLSV

SEQ ID NO: 111 - protein, 110 aa, Streptococcus equi subsp. equi
LPEKGLNGENQKEPEQGERGEAGPPLSGLSGNNQGRPSLPGLNGENQKEPEQGERGEAGPPSTPNLEGNNRKNPLKGLDGENKPKEDLDGKGLSGENDESPKLKDEHPYN

SEQ ID NO: 112 - protein, 110 aa, Streptococcus equi subsp. zooepidemicus
LPEKGLNGENQKEPEQGERGEAGPPSTPNLEGNNRKNPLKGLDGENKPKEDLDGKGLSGENDESPKLKDEHPYNHGRRDGYRVGYEDGYGGKKHKGDYPKRFDESSPKEY

SEQ ID NO: 113 - protein, 20 aa, Homo sapiens
RFKQDGGWSHWSPWSSCSVT

SEQ ID NO: 114 - protein, 40 aa, Homo sapiens
GPAGAPGTPGPQGIAGQRGVVGLPGQRGERGFPGLPGPSG

SEQ ID NO: 115 - protein, 12 aa, Homo sapiens
TLQPVYEYMVGV

SEQ ID NO: 116 - protein, 15 aa, Homo sapiens
TGLPVGVGYVVTVLT

SEQ ID NO: 117 - protein, 36 aa, Streptococcus pyogenes
TEVYGNQQNPVDIDKKLPNETGFSGNMVETEDTKEP

SEQ ID NO: 118 - protein, 37 aa, Streptococcus pyogenes
EVLMGGQSESVEFTKDTQTGMSGQTTPQVETEDTKEP

SEQ ID NO: 119 - protein, 37 aa, Streptococcus pyogenes
GVLMGGQSESVEFTKDTQTGMSGQTTPQVETEDTKEP

SEQ ID NO: 120 - protein, 51 aa, Streptococcus pyogenes
GVLMGGQSESVEFTKDTQTGMSGFSETVTIIEDTRPKLVFHFDNNEPKVEE

SEQ ID NO: 121 - protein, 39 aa, Streptococcus pyogenes
VSTQENKDPIVDITEDTQPGMSGSNDATVVEEDTTPQRP

SEQ ID NO: 122 - protein, 39 aa, Streptococcus pyogenes
DVLVGGQSDPIDITEDTQPGMSGSNDATVVEEDTVPKRP

SEQ ID NO: 123 - protein, 82 aa, Streptococcus pyogenes
DILVGGQSDPIDITEDTQPGMSGSNDATVIEEDTKPKRFFHFDNEPQAPEKPKEQPSLSLPQAPVYKAAHHLPASGDKREAS

SEQ ID NO: 124 - protein, 36 aa, Streptococcus pyogenes
REVITQQGPNLEIEETLPLESGASGGTTTVEDSRPV

SEQ ID NO: 125 - protein, 36 aa, Streptococcus pyogenes
YKPTKGSGQVIDIEEKLPDEQGHSGSTTEIEDSKPS

SEQ ID NO: 126 - protein, 37 aa, Streptococcus pyogenes
DVIIGGQGEVVDTTEDTQSGMTGHSGSTTEIEDSKSS

SEQ ID NO: 127 - protein, 47 aa, Streptococcus pyogenes
DVIIGGQGQVVETTEDTQTGMHGDSGCKTEVEDTKLVQLFHFDNKEP

SEQ ID NO: 128 - protein, 38 aa, Streptococcus equi
KPGQTGGQGPVIETTEDTQKGMSGQSGGTIESENTKKP

SEQ ID NO: 129 - protein, 37 aa, Streptococcus equi
EVMIGGQGQTIETTEDTQKGMSGQSGGTIESEDTKKP

SEQ ID NO: 130 - protein, 37 aa, Streptococcus equi
EVMIGGQGQIIDFSENTQSGMSGQSGDTTVIEDTKKS

SEQ ID NO: 131 - protein, 38 aa, Streptococcus equi
EIIIGGQGQIIDFSEDTQPGMSGQSGGTTIVEDTKKPT

SEQ ID NO: 132 - protein, 47 aa, Streptococcus dysgalactiae
GPTEGENNLGGQSEEITITEDSQSGMSGQNPGSGNETVVEDTQTSQE

SEQ ID NO: 133 - protein, 39 aa, Streptococcus dysgalactiae
DIVLGGPGQVIDFTEDSQPGMSGNNSHTITEDSKPSQED

SEQ ID NO: 134 - protein, 43 aa, Streptococcus dysgalactiae
EVIIGGQGQVIDFTEDTQSGMSGDNSHTDGTVLEEDSKPSQED

SEQ ID NO: 135 - protein, 39 aa, Streptococcus dysgalactiae
EVIIGGQGQVIDFTEDTQTGMSGAGQVESPTITEETHKP

SEQ ID NO: 136 - protein, 52 aa, Streptococcus dysgalactiae
EIIMGGQSDPIDMVEDTLPGMSGSNEATVVEEDTRPKLQFHFDNEEPVPATV

SEQ ID NO: 137 - protein, 37 aa, Streptococcus dysgalactiae
TKREVIIQQGPILGLEETLPTEEHQSGDTTTIEDTRP

SEQ ID NO: 138 - protein, 36 aa, Streptococcus dysgalactiae
DKPITEASQSIDFEETLPTEQGQSGSTTEVEDTKGP

SEQ ID NO: 139 - protein, 36 aa, Streptococcus dysgalactiae
EVIIGGQGEIVDIEENLPTEQGQSGSTTEVEDTKGP

SEQ ID NO: 140 - protein, 83 aa, Streptococcus dysgalactiae
EVIIGGQGEVVDIEESLPTEQGQSGSTTEVEDSKPKLSIHFDNEWPKEDKPQLPAVEKPKTKESLPAAGEAEHVLSTIVGAMI

SEQ ID NO: 141 - protein, 39 aa, Staphylococcus aureus
GPIIQNNKFEYKEDTIKETLTGQYDKNLVTTVEEEYDSS

SEQ ID NO: 142 - protein, 29 aa, Staphylococcus aureus
IDFEESTHENSKHHADVVEYEEDTNPGGG

SEQ ID NO: 143 - protein, 34 aa, Staphylococcus aureus
QVTTESNLVEFDEESTKGIVTGAVSDHTTVEDTK

SEQ ID NO: 144 - protein, 38 aa, Staphylococcus aureus
KYEQGGNIVDIDFDSVPQIHGQNKGNQSFEEDTEKDKP

SEQ ID NO: 145 - protein, 38 aa, Staphylococcus aureus
KYEHGGNIIDIDFDSVPHIHGFNKHTEIIEEDTNKDKP

SEQ ID NO: 146 - protein, 36 aa, Staphylococcus aureus
SYQFGGHNSVDFEEDTLPKVSGQNEGQQTIEEDTTP

SEQ ID NO: 147 - protein, 60 aa, Borrelia burgdorferi
SGELEEPIESNEIDLTIDSDLRPKSSLQGIAGSNSISYTDEIEEEDYDQYYLDEYDEEDE

SEQ ID NO: 148 - DNA, 21 bp, Streptococcus pyogenes
accgaagtgtatggcaaccag

SEQ ID NO: 149 - DNA, 21 bp, Streptococcus pyogenes
gtggatattgataaaaaactg

SEQ ID NO: 150 - DNA, 21 bp, Streptococcus pyogenes
ccgaacgaaaccggctttagc

SEQ ID NO: 151 - DNA, 21 bp, Streptococcus pyogenes
atggtggaaaccgaagatacc

SEQ ID NO: 152 - DNA, 21 bp, Streptococcus pyogenes
gaagtgctgatgggcggccag

SEQ ID NO: 153 - DNA, 21 bp, Streptococcus pyogenes
gtggaatttaccaaagatacc

SEQ ID NO: 154 - DNA, 21 bp, Streptococcus pyogenes
accggcatgagcggccagacc

SEQ ID NO: 155 - DNA, 21 bp, Streptococcus pyogenes
caggtggaaaccgaagatacc

SEQ ID NO: 156 - DNA, 21 bp, Streptococcus pyogenes
ggcgtgctgatgggcggccag

SEQ ID NO: 157 - DNA, 21 bp, Streptococcus pyogenes
accggcatgagcggctttagc

SEQ ID NO: 158 - DNA, 21 bp, Streptococcus pyogenes
gtgaccattattgaagatacc

SEQ ID NO: 159 - DNA, 21 bp, Streptococcus pyogenes
ctggtgtttcattttgataac

SEQ ID NO: 160 - DNA, 21 bp, Streptococcus pyogenes
gtgagcacccaggaaaacaaa

SEQ ID NO: 161 - DNA, 21 bp, Streptococcus pyogenes
gtggatattaccgaagatacc

SEQ ID NO: 162 - DNA, 21 bp, Streptococcus pyogenes
ccgggcatgagcggcagcaac

SEQ ID NO: 163 - DNA, 21 bp, Streptococcus pyogenes
accgtggtggaagaagatacc

SEQ ID NO: 164 - DNA, 21 bp, Streptococcus pyogenes
gatgtgctggtgggcggccag

SEQ ID NO: 165 - DNA, 21 bp, Streptococcus pyogenes
attgatattaccgaagatacc

SEQ ID NO: 166 - DNA, 21 bp, Streptococcus pyogenes
gatattctggtgggcggccag

SEQ ID NO: 167 - DNA, 21 bp, Streptococcus pyogenes
accgtgattgaagaagatacc

SEQ ID NO: 168 - DNA, 21 bp, Streptococcus pyogenes
cgcttttttcattttgataac

SEQ ID NO: 169 - DNA, 21 bp, Streptococcus pyogenes
cgcgaagtgattacccagcag

SEQ ID NO: 170 - DNA, 21 bp, Streptococcus pyogenes
aacctggaaattgaagaaacc

SEQ ID NO: 171 - DNA, 21 bp, Streptococcus pyogenes
ccgctggaaagcggcgcgagc

SEQ ID NO: 172 - DNA, 21 bp, Streptococcus pyogenes
accaccaccgtggaagatagc

SEQ ID NO: 173 - DNA, 21 bp, Streptococcus pyogenes
tataaaccgaccaaaggcagc

SEQ ID NO: 174 - DNA, 21 bp, Streptococcus pyogenes
gtgattgatattgaagaaaaa

SEQ ID NO: 175 - DNA, 21 bp, Streptococcus pyogenes
ccggatgaacagggccatagc

SEQ ID NO: 176 - DNA, 21 bp, Streptococcus pyogenes
accaccgaaattgaagatagc

SEQ ID NO: 177 - DNA, 21 bp, Streptococcus pyogenes
gatgtgattattggcggccag

SEQ ID NO: 178 - DNA, 21 bp, Streptococcus pyogenes
gtggataccaccgaagatacc

SEQ ID NO: 179 - DNA, 21 bp, Streptococcus pyogenes
agcggcatgaccggccatagc

SEQ ID NO: 180 - DNA, 21 bp, Streptococcus pyogenes
gtggaaaccaccgaagatacc

SEQ ID NO: 181 - DNA, 21 bp, Streptococcus pyogenes
accggcatgcatggcgatagc

SEQ ID NO: 182 - DNA, 21 bp, Streptococcus pyogenes
aaaaccgaagtggaagatacc

SEQ ID NO: 183 - DNA, 21 bp, Streptococcus pyogenes
cagctgtttcattttgataac

SEQ ID NO: 184 - DNA, 21 bp, Streptococcus equi
ccgggccagaccggcggccag

SEQ ID NO: 185 - DNA, 21 bp, Streptococcus equi
attgaaaccaccgaagatacc

SEQ ID NO: 186 - DNA, 21 bp, Streptococcus equi
aaaggcatgagcggccagagc

SEQ ID NO: 187 - DNA, 21 bp, Streptococcus equi
accattgaaagcgaaaacacc

SEQ ID NO: 188 - DNA, 21 bp, Streptococcus equi
gaagtgatgattggcggccag

SEQ ID NO: 189 - DNA, 21 bp, Streptococcus equi
accattgaaagcgaagatacc

SEQ ID NO: 190 - DNA, 21 bp, Streptococcus equi
attgattttagcgaaaacacc

SEQ ID NO: 191 - DNA, 21 bp, Streptococcus equi
agcggcatgagcggccagagc

SEQ ID NO: 192 - DNA, 21 bp, Streptococcus equi
accaccgtgattgaagatacc

SEQ ID NO: 193 - DNA, 21 bp, Streptococcus equi
gaaattattattggcggccag

SEQ ID NO: 194 - DNA, 21 bp, Streptococcus equi
attgattttagcgaagatacc

SEQ ID NO: 195 - DNA, 21 bp, Streptococcus equi
ccgggcatgagcggccagagc

SEQ ID NO: 196 - DNA, 21 bp, Streptococcus equi
accaccattgtggaagatacc

SEQ ID NO: 197 - DNA, 21 bp, Streptococcus dysgalactiae
gaaaacaacctgggcggccag

SEQ ID NO: 198 - DNA, 21 bp, Streptococcus dysgalactiae
attaccattaccgaagatagc

SEQ ID NO: 199 - DNA, 21 bp, Streptococcus dysgalactiae
agcggcatgagcggccagaac

SEQ ID NO: 200 - DNA, 21 bp, Streptococcus dysgalactiae
gaaaccgtggtggaagatacc

SEQ ID NO: 201 - DNA, 21 bp, Streptococcus dysgalactiae
gatattgtgctgggcggcccg

SEQ ID NO: 202 - DNA, 21 bp, Streptococcus dysgalactiae
attgattttaccgaagatagc

SEQ ID NO: 203 - DNA, 21 bp, Streptococcus dysgalactiae
ccgggcatgagcggcaacaac

SEQ ID NO: 204 - DNA, 21 bp, Streptococcus dysgalactiae
cataccattaccgaagatagc

SEQ ID NO: 205 - DNA, 21 bp, Streptococcus dysgalactiae
gaagtgattattggcggccag

SEQ ID NO: 206 - DNA, 21 bp, Streptococcus dysgalactiae
attgattttaccgaagatacc

SEQ ID NO: 207 - DNA, 21 bp, Streptococcus dysgalactiae
agcggcatgagcggcgataac

SEQ ID NO: 208 - DNA, 21 bp, Streptococcus dysgalactiae
accgtgctggaagaagatagc

SEQ ID NO: 209 - DNA, 21 bp, Streptococcus dysgalactiae
accggcatgagcggcgcgggc

SEQ ID NO: 210 - DNA, 21 bp, Streptococcus dysgalactiae
ccgaccattaccgaagaaacc

SEQ ID NO: 211 - DNA, 21 bp, Streptococcus dysgalactiae
gaaattattatgggcggccag

SEQ ID NO: 212 - DNA, 21 bp, Streptococcus dysgalactiae
attgatatggtggaagatacc

SEQ ID NO: 213 - DNA, 21 bp, Streptococcus dysgalactiae
ccgggcatgagcggcagcaac

SEQ ID NO: 214 - DNA, 21 bp, Streptococcus dysgalactiae
accgtggtggaagaagatacc

SEQ ID NO: 215 - DNA, 21 bp, Streptococcus dysgalactiae
ctgcagtttcattttgataac

SEQ ID NO: 216 - DNA, 21 bp, Streptococcus dysgalactiae
gaagtgattattcagcagggc

SEQ ID NO: 217 - DNA, 21 bp, Streptococcus dysgalactiae
attctgggcctggaagaaacc

SEQ ID NO: 218 - DNA, 21 bp, Streptococcus dysgalactiae
ccgaccgaagaacatcagagc

SEQ ID NO: 219 - DNA, 21 bp, Streptococcus dysgalactiae
accaccaccattgaagatacc

SEQ ID NO: 220 - DNA, 21 bp, Streptococcus dysgalactiae
gataaaccgattaccgaagcg

SEQ ID NO: 221 - DNA, 21 bp, Streptococcus dysgalactiae
agcattgattttgaagaaacc

SEQ ID NO: 222 - DNA, 21 bp, Streptococcus dysgalactiae
ccgaccgaacagggccagagc

SEQ ID NO: 223 - DNA, 21 bp, Streptococcus dysgalactiae
accaccgaagtggaagatacc

SEQ ID NO: 224 - DNA, 21 bp, Streptococcus dysgalactiae
attgtggatattgaagaaaac

SEQ ID NO: 225 - DNA, 21 bp, Streptococcus dysgalactiae
gtggtggatattgaagaaagc

SEQ ID NO: 226 - DNA, 21 bp, Streptococcus dysgalactiae
accaccgaagtggaagatagc

SEQ ID NO: 227 - DNA, 21 bp, Streptococcus dysgalactiae
ctgagcattcattttgataac

SEQ ID NO: 228 - DNA, 21 bp, Staphylococcus aureus
ggtccaattattcaaaataat

SEQ ID NO: 229 - DNA, 21 bp, Staphylococcus aureus
tttgaatataaagaagataca

SEQ ID NO: 230 - DNA, 21 bp, Staphylococcus aureus
gaaacattaacaggtcaatat

SEQ ID NO: 231 - DNA, 21 bp, Staphylococcus aureus
acaacagttgaagaagaatat

SEQ ID NO: 232 - DNA, 18 bp, Staphylococcus aureus
attgattttgaagaatca

SEQ ID NO: 233 - DNA, 21 bp, Staphylococcus aureus
gaaaattcaaaacatcatgca

SEQ ID NO: 234 - DNA, 21 bp, Staphylococcus aureus
gttgaatatgaagaagataca

SEQ ID NO: 235 - DNA, 21 bp, Staphylococcus aureus
caagttacaacagaatcaaat

SEQ ID NO: 236 - DNA, 21 bp, Staphylococcus aureus
gttgaatttgatgaagaatca

SEQ ID NO: 237 - DNA, 21 bp, Staphylococcus aureus
ggtattgttacaggtgcagtt

SEQ ID NO: 238 - DNA, 21 bp, Staphylococcus aureus
catacaacagttgaagataca

SEQ ID NO: 239 - DNA, 21 bp, Staphylococcus aureus
aaatatgaacaaggtggtaat

SEQ ID NO: 240 - DNA, 21 bp, Staphylococcus aureus
gttgatattgattttgattca

SEQ ID NO: 241 - DNA, 21 bp, Staphylococcus aureus
ccacaaattcatggtcaaaat

SEQ ID NO: 242 - DNA, 21 bp, Staphylococcus aureus
caatcatttgaagaagataca

SEQ ID NO: 243 - DNA, 21 bp, Staphylococcus aureus
aaatatgaacatggtggtaat

SEQ ID NO: 244 - DNA, 21 bp, Staphylococcus aureus
attgatattgattttgattca

SEQ ID NO: 245 - DNA, 21 bp, Staphylococcus aureus
ccacatattcatggttttaat

SEQ ID NO: 246 - DNA, 21 bp, Staphylococcus aureus
gaaattattgaagaagataca

SEQ ID NO: 247 - DNA, 21 bp, Staphylococcus aureus
tcatatcaatttggtggtcat

SEQ ID NO: 248 - DNA, 21 bp, Staphylococcus aureus
gttgattttgaagaagataca

SEQ ID NO: 249 - DNA, 21 bp, Staphylococcus aureus
ccaaaagtttcaggtcaaaat

SEQ ID NO: 250 - DNA, 21 bp, Staphylococcus aureus
caaacaattgaagaagataca

SEQ ID NO: 251 - DNA, 18 bp, Borrelia burgdorferi
gaaccgattgaaagcaac

SEQ ID NO: 252 - DNA, 21 bp, Borrelia burgdorferi
attgatctgaccattgatagc

SEQ ID NO: 253 - DNA, 21 bp, Borrelia burgdorferi
cagggcattgcgggcagcaac

SEQ ID NO: 254 - DNA, 21 bp, Borrelia burgdorferi
gaaattgaagaagaagattat

SEQ ID NO: 255 - DNA, 33 bp, Mycobacterium tuberculosis
ttcgagtggtacgaccagtcgggcctgtcggtg

SEQ ID NO: 256 - DNA, 33 bp, Mycobacterium tuberculosis
ttcgagtggtactaccagtcgggcctgtcgatc

SEQ ID NO: 257 - DNA, 33 bp, Mycobacterium tuberculosis
ttcgaggagtactaccagtcgggcctgtcggtg

SEQ ID NO: 258 - DNA, 330 bp, Streptococcus equi subsp. equi
ctgccggaaaaaggcctgaacggcgaaaaccagaaagaaccggaacagggcgaacgcggcgaagcgggcccgccgctgagcggcctgagcggcaacaaccagggccgcccgagcctgccgggcctgaacggcgaaaaccagaaagaaccggaacagggcgaacgcggcgaagcgggcccgccgagcaccccgaacctggaaggcaacaaccgcaaaaacccgctgaaaggcctggatggcgaaaacaaaccgaaagaagatctggatggcaaaggcctgagcggcgaaaacgatgaaagcccgaaactgaaagatgaacatccgtataac

SEQ ID NO: 259 - DNA, 330 bp, Streptococcus equi subsp. zooepidemicus
ctgccggaaaaaggcctgaacggcgaaaaccagaaagaaccggaacagggcgaacgcggcgaagcgggcccgccgagcaccccgaacctggaaggcaacaaccgcaaaaacccgctgaaaggcctggatggcgaaaacaaaccgaaagaagatctggatggcaaaggcctgagcggcgaaaacgatgaaagcccgaaactgaaagatgaacatccgtataaccatggccgccgcgatggctatcgcgtgggctatgaagatggctatggcggcaaaaaacataaaggcgattatccgaaacgctttgatgaaagcagcccgaaagaatat

SEQ ID NO: 260 - DNA, 60 bp, Homo sapiens
aggttcaagcaggacggcggctggagccactggagcccctggagcagctgcagcgtgacc

SEQ ID NO: 261 - DNA, 120 bp, Homo sapiens
ggccccgccggcgcccccggcacccccggcccccagggcatcgccggccagaggggcgtggtgggcctgcccggccagaggggcgagaggggcttccccggcctgcccggccccagcggc

SEQ ID NO: 262 - DNA, 36 bp, Homo sapiens
accctgcagcccgtgtacgagtacatggtgggcgtg

SEQ ID NO: 263 - DNA, 45 bp, Homo sapiens
accggcctgcccgtgggcgtgggctacgtggtgaccgtgctgacc

SEQ ID NO: 264 - DNA, 108 bp, Streptococcus pyogenes
accgaagtgtatggcaaccagcagaacccggtggatattgataaaaaactgccgaacgaaaccggctttagcggcaacatggtggaaaccgaagataccaaagaaccg

SEQ ID NO: 265 - DNA, 111 bp, Streptococcus pyogenes
gaagtgctgatgggcggccagagcgaaagcgtggaatttaccaaagatacccagaccggcatgagcggccagaccaccccgcaggtggaaaccgaagataccaaagaaccg

SEQ ID NO: 266 - DNA, 111 bp, Streptococcus pyogenes
ggcgtgctgatgggcggccagagcgaaagcgtggaatttaccaaagatacccagaccggcatgagcggccagaccaccccgcaggtggaaaccgaagataccaaagaaccg

SEQ ID NO: 267 - DNA, 153 bp, Streptococcus pyogenes
ggcgtgctgatgggcggccagagcgaaagcgtggaatttaccaaagatacccagaccggcatgagcggctttagcgaaaccgtgaccattattgaagatacccgcccgaaactggtgtttcattttgataacaacgaaccgaaagtggaagaa

SEQ ID NO: 268 - DNA, 117 bp, Streptococcus pyogenes
gtgagcacccaggaaaacaaagatccgattgtggatattaccgaagatacccagccgggcatgagcggcagcaacgatgcgaccgtggtggaagaagataccaccccgcagcgcccg

SEQ ID NO: 269 - DNA, 117 bp, Streptococcus pyogenes
gatgtgctggtgggcggccagagcgatccgattgatattaccgaagatacccagccgggcatgagcggcagcaacgatgcgaccgtggtggaagaagataccgtgccgaaacgcccg

SEQ ID NO: 270 - DNA, 246 bp, Streptococcus pyogenes
gatattctggtgggcggccagagcgatccgattgatattaccgaagatacccagccgggcatgagcggcagcaacgatgcgaccgtgattgaagaagataccaaaccgaaacgcttttttcattttgataacgaaccgcaggcgccggaaaaaccgaaagaacagccgagcctgagcctgccgcaggcgccggtgtataaagcggcgcatcatctgccggcgagcggcgataaacgcgaagcgagc

SEQ ID NO: 271 - DNA, 108 bp, Streptococcus pyogenes
cgcgaagtgattacccagcagggcccgaacctggaaattgaagaaaccctgccgctggaaagcggcgcgagcggcggcaccaccaccgtggaagatagccgcccggtg

SEQ ID NO: 272 - DNA, 108 bp, Streptococcus pyogenes
tataaaccgaccaaaggcagcggccaggtgattgatattgaagaaaaactgccggatgaacagggccatagcggcagcaccaccgaaattgaagatagcaaaccgagc

SEQ ID NO: 273 - DNA, 111 bp, Streptococcus pyogenes
gatgtgattattggcggccagggcgaagtggtggataccaccgaagatacccagagcggcatgaccggccatagcggcagcaccaccgaaattgaagatagcaaaagcagc

SEQ ID NO: 274 - DNA, 141 bp, Streptococcus pyogenes
gatgtgattattggcggccagggccaggtggtggaaaccaccgaagatacccagaccggcatgcatggcgatagcggctgcaaaaccgaagtggaagataccaaactggtgcagctgtttcattttgataacaaagaaccg

SEQ ID NO: 275 - DNA, 114 bp, Streptococcus equi
aaaccgggccagaccggcggccagggcccggtgattgaaaccaccgaagatacccagaaaggcatgagcggccagagcggcggcaccattgaaagcgaaaacaccaaaaaaccg

SEQ ID NO: 276 - DNA, 111 bp, Streptococcus equi
gaagtgatgattggcggccagggccagaccattgaaaccaccgaagatacccagaaaggcatgagcggccagagcggcggcaccattgaaagcgaagataccaaaaaaccg

SEQ ID NO: 277 - DNA, 111 bp, Streptococcus equi
gaagtgatgattggcggccagggccagattattgattttagcgaaaacacccagagcggcatgagcggccagagcggcgataccaccgtgattgaagataccaaaaaaagc

SEQ ID NO: 278 - DNA, 114 bp, Streptococcus equi
gaaattattattggcggccagggccagattattgattttagcgaagatacccagccgggcatgagcggccagagcggcggcaccaccattgtggaagataccaaaaaaccgacc

SEQ ID NO: 279 - DNA, 141 bp, Streptococcus dysgalactiae
ggtccaacagaaggtgaaaataatttaggtggtcaatcagaagaaattacaattacagaagattcacaatcaggtatgtcaggtcaaaatccaggttcaggtaatgaaacagttgttgaagatacacaaacatcacaagaa

SEQ ID NO: 280 - DNA, 117 bp, Streptococcus dysgalactiae
gatattgttttaggtggtccaggtcaagttattgattttacagaagattcacaaccaggtatgtcaggtaataattcacatacaattacagaagattcaaaaccatcacaagaagat

SEQ ID NO: 281 - DNA, 129 bp, Streptococcus dysgalactiae
gaagttattattggtggtcaaggtcaagttattgattttacagaagatacacaatcaggtatgtcaggtgataattcacatacagatggtacagttttagaagaagattcaaaaccatcacaagaagat

SEQ ID NO: 282 - DNA, 117 bp, Streptococcus dysgalactiae
gaagttattattggtggtcaaggtcaagttattgattttacagaagatacacaaacaggtatgtcaggtgcaggtcaagttgaatcaccaacaattacagaagaaacacataaacca

SEQ ID NO: 283 - DNA, 156 bp, Streptococcus dysgalactiae
gaaattattatgggtggtcaatcagatccaattgatatggttgaagatacattaccaggtatgtcaggttcaaatgaagcaacagttgttgaagaagatacaagaccaaaattacaatttcattttgataatgaagaaccagttccagcaacagtt

SEQ ID NO: 284 - DNA, 111 bp, Streptococcus dysgalactiae
acaaaaagagaagttattattcaacaaggtccaattttaggtttagaagaaacattaccaacagaagaacatcaatcaggtgatacaacaacaattgaagatacaagacca

SEQ ID NO: 285 - DNA, 108 bp, Streptococcus dysgalactiae
gataaaccaattacagaagcatcacaatcaattgattttgaagaaacattaccaacagaacaaggtcaatcaggttcaacaacagaagttgaagatacaaaaggtcca

SEQ ID NO: 286 - DNA, 108 bp, Streptococcus dysgalactiae
gaagttattattggtggtcaaggtgaaattgttgatattgaagaaaatttaccaacagaacaaggtcaatcaggttcaacaacagaagttgaagatacaaaaggtcca

SEQ ID NO: 287 - DNA, 249 bp, Streptococcus dysgalactiae
gaagttattattggtggtcaaggtgaagttgttgatattgaagaatcattaccaacagaacaaggtcaatcaggttcaacaacagaagttgaagattcaaaaccaaaattatcaattcattttgataatgaatggccaaaagaagataaaccacaattaccagcagttgaaaaaccaaaaacaaaagaatcattaccagcagcaggtgaagcagaacatgttttatcaacaattgttggtgcaatgatt

SEQ ID NO: 288 - DNA, 117 bp, Staphylococcus aureus
ggtccaattattcaaaataataaatttgaatataaagaagatacaattaaagaaacattaacaggtcaatatgataaaaatttagttacaacagttgaagaagaatatgattcatca

SEQ ID NO: 289 - DNA, 87 bp, Staphylococcus aureus
attgattttgaagaatcaacacatgaaaattcaaaacatcatgcagatgttgttgaatatgaagaagatacaaatccaggtggtggt

SEQ ID NO: 290 - DNA, 102 bp, Staphylococcus aureus
caagttacaacagaatcaaatttagttgaatttgatgaagaatcaacaaaaggtattgttacaggtgcagtttcagatcatacaacagttgaagatacaaaa

SEQ ID NO: 291 - DNA, 114 bp, Staphylococcus aureus
aaatatgaacaaggtggtaatattgttgatattgattttgattcagttccacaaattcatggtcaaaataaaggtaatcaatcatttgaagaagatacagaaaaagataaacca

SEQ ID NO: 292 - DNA, 114 bp, Staphylococcus aureus
aaatatgaacatggtggtaatattattgatattgattttgattcagttccacatattcatggttttaataaacatacagaaattattgaagaagatacaaataaagataaacca

SEQ ID NO: 293 - DNA, 108 bp, Staphylococcus aureus
tcatatcaatttggtggtcataattcagttgattttgaagaagatacattaccaaaagtttcaggtcaaaatgaaggtcaacaaacaattgaagaagatacaacacca

SEQ ID NO: 294 - DNA, 180 bp, Borrelia burgdorferi
agcggcgaactggaagaaccgattgaaagcaacgaaattgatctgaccattgatagcgatctgcgcccgaaaagcagcctgcagggcattgcgggcagcaacagcattagctataccgatgaaattgaagaagaagattatgatcagtattatctggatgaatatgatgaagaagatgaa

SEQ ID NO: 295 - protein, 38 aa, Staphylococcus aureus
CGGGQVTTESNLVEFDEESTKGIVTGAVSDHTTVEDTK

SEQ ID NO: 296 - protein, 38 aa, Artificial Sequence
CGSEQEDLTGTKVDFGETIVVNEATETVTSGSTHGTKV